European Patent Application EP 4 789 681 A1, published August 12, 2026. Title: 经糖基修饰的融合蛋白、核酸分子、表达载体、宿主细胞及应用. Applicant: 凯米生物医药（成都）有限公司. Application CN. The sequence listing filed with the application follows.

SEQUENCE LISTING (16 sequences)

SEQ ID NO: 1 - protein, 232 aa, Mus musculus
VDKKIVPRDCGCKPCICTVPEVSSVFIFPPKPKDVLTITLTPKVTCVVVDISKDDPEVQFSWFVDDVEVHTAQTQPREEQFNSTFRSVSELPIMHQDWLNGKEFKCRVNSAAFPAPIEKTISKTKGRPKAPQVYTIPPPKEQMAKDKVSLTCMITDFFPEDITVEWQWNGQPAENYKNTQPIMDTDGSYFVYSKLNVQKSNWEAGNTFTCSVLHEGLHNHHTEKSLSHSPGL

SEQ ID NO: 2 - protein, 232 aa, synthetic construct
VDKKIVPADCGCAPCICAVPEVSSVFIFPPKPKDVLTITLTPKVTCVVVDISKDDPEVQFSWFVDDVEVHTAQTQPREEQFNSTFRSVSELPIMHQDWLNGKEFKCRVNSAAFPAPIEKTISKTKGRPKAPQVYTIPPPKEQMAKDKVSLTCMITDFFPEDITVEWQWNGQPAENYKNTQPIMDTDGSYFVYSKLNVQKSNWEAGNTFTCSVLHEGLHNHHTEKSLSHSPGL

SEQ ID NO: 3 - protein, 232 aa, synthetic construct
VDKKIVPADCGCAPCICAVPEVSSVFIFPPKPKDVLTITLTPKVTCVVVDISKDDPEVQFSWFVDDVEVHTAQTQPREEQFNSTFRSVSELPIMHQDWLNGKEFKCRVNSAAFPLPEEKTISKTKGRPKAPQVYTIPPPKEQMAKDKVSLTCMITDFFPEDITVEWQWNGQPAENYKNTQPIMDTDGSYFVYSKLNVQKSNWEAGNTFTCSVLHEGLHNHHTEKSLSHSPGL

SEQ ID NO: 4 - protein, 644 aa, synthetic construct
SYYHHHHHHDYDIPTTENLYFQGAMDPEFKGLRRRMKKWSSKPRKGMGTNLSVPNPLGFFPDHQLDPVFGANSNNPDWDFNPIKDHWPAANQVGVGAFGPGFTPPHGGVLGWSPQAQGMLTPVSTIPPPASANRQSGRQPTPISPPLRDSHPQAMQWNSTAFHQALQDPRVRGLYFPAGGSSSGTVNPAPNIASHISSISARTGDPVTNMDIDPYKEFGATVELLSFLPSDFFPSVRDLLDTASALYREALESPEHCSPHHTALRQAILCWGELMTLATWVGNNLEDPASRDLVVNYVNTNMGLKIRQLLWFHISCLTFGRETVLEYLVSFGVWIRTPPAYRPPNAPILSTLPETTVVRRRDRGRSPRRRTPSPRRRRSQSPRRRRSQSRESQCVRPQGGGSVDKKIVPADCGCAPCICAVPEVSSVFIFPPKPKDVLTITLTPKVTCVVVDISKDDPEVQFSWFVDDVEVHTAQTQPREEQFNSTFRSVSELPIMHQDWLNGKEFKCRVNSAAFPLPEEKTISKTKGRPKAPQVYTIPPPKEQMAKDKVSLTCMITDFFPEDITVEWQWNGQPAENYKNTQPIMDTDGSYFVYSKLNVQKSNWEAGNTFTCSVLHEGLHNHHTEKSLSHSPGLQSLSRSTRGS

SEQ ID NO: 5 - protein, 449 aa, synthetic construct
SYYHHHHHHDYDIPTTENLYFQGAMDPEFKGLRRRMKKWSSKPRKGMGTNLSVPNPLGFFPDHQLDPVFGANSNNPDWDFNPIKDHWPAANQVGVGAFGPGFTPPHGGVLGWSPQAQGMLTPVSTIPPPASANRQSGRQPTPISPPLRDSHPQAMQWNSTAFHQALQDPRVRGLYFPAGGSSSGTVNPAPNIASHISSISARTGDPVTNVRPQGGGSVDKKIVPADCGCAPCICAVPEVSSVFIFPPKPKDVLTITLTPKVTCVVVDISKDDPEVQFSWFVDDVEVHTAQTQPREEQFNSTFRSVSELPIMHQDWLNGKEFKCRVNSAAFPAPIEKTISKTKGRPKAPQVYTIPPPKEQMAKDKVSLTCMITDFFPEDITVEWQWNGQPAENYKNTQPIMDTDGSYFVYSKLNVQKSNWEAGNTFTCSVLHEGLHNHHTEKSLSHSPGL

SEQ ID NO: 6 - protein, 449 aa, synthetic construct
SYYHHHHHHDYDIPTTENLYFQGAMDPEFKGLRRRMKKWSSKPRKGMGTNLSVPNPLGFFPDHQLDPVFGANSNNPDWDFNPIKDHWPAANQVGVGAFGPGFTPPHGGVLGWSPQAQGMLTPVSTIPPPASANRQSGRQPTPISPPLRDSHPQAMQWNSTAFHQALQDPRVRGLYFPAGGSSSGTVNPAPNIASHISSISARTGDPVTNVRPQGGGSVDKKIVPADCGCAPCICAVPEVSSVFIFPPKPKDVLTITLTPKVTCVVVDISKDDPEVQFSWFVDDVEVHTAQTQPREEQFNSTFRSVSELPIMHQDWLNGKEFKCRVNSAAFPLPEEKTISKTKGRPKAPQVYTIPPPKEQMAKDKVSLTCMITDFFPEDITVEWQWNGQPAENYKNTQPIMDTDGSYFVYSKLNVQKSNWEAGNTFTCSVLHEGLHNHHTEKSLSHSPGL

SEQ ID NO: 7 - protein, 644 aa, synthetic construct
SYYHHHHHHDYDIPTTENLYFQGAMDPEFKGLRRRMKKWSSKPRKGMGTNLSVPNPLGFFPDHQLDPVFGANSNNPDWDFNPIKDHWPAANQVGVGAFGPGFTPPHGGVLGWSPQAQGMLTPVSTIPPPASANRQSGRQPTPISPPLRDSHPQAMQWNSTAFHQALQDPRVRGLYFPAGGSSSGTVNPAPNIASHISSISARTGDPVTNMDIDPYKEFGATVELLSFLPSDFFPSVRDLLDTASALYREALESPEHCSPHHTALRQAILCWGELMTLATWVGNNLEDPASRDLVVNYVNTNMGLKIRQLLWFHISCLTFGRETVLEYLVSFGVWIRTPPAYRPPNAPILSTLPETTVVRRRDRGRSPRRRTPSPRRRRSQSPRRRRSQSRESQCVRPQGGGSVDKKIVPADCGCAPCICAVPEVSSVFIFPPKPKDVLTITLTPKVTCVVVDISKDDPEVQFSWFVDDVEVHTAQTQPREEQFNSTFRSVSELPIMHQDWLNGKEFKCRVNSAAFPAPIEKTISKTKGRPKAPQVYTIPPPKEQMAKDKVSLTCMITDFFPEDITVEWQWNGQPAENYKNTQPIMDTDGSYFVYSKLNVQKSNWEAGNTFTCSVLHEGLHNHHTEKSLSHSPGLQSLSRSTRGS

SEQ ID NO: 8 - protein, 592 aa, synthetic construct
KELKFVTLVFRHGDRSPIDTFPTDPIKESSWPQGFGQLTQLGMEQHYELGEYIRKRYRKFLNESYKHEQVYIRSTDVDRTLMSAMTNLAALFPPEGVSIWNPILLWQPIPVHTVPLSEDQLLYLPFRNCPRFQELESETLKSEEFQKRLHPYKDFIATLGKLSGLHGQDLFGIWSKVYDPLYCESVHNFTLPSWATEDTMTKLRELSELSLLSLYGIHKQKEKSRLQGGVLVNEILNHMKRATQIPSYKKLIMYSAHDTTVSGLQMALDVYNGLLPPYASCHLTELYFEKGEYFVEMYYRNETQHEPYPLMLPGCSPSCPLERFAELVGPVIPQDWSTECMTTNSHQGTEDSTDSRGGGSVDKKIVPADCGCAPCICAVPEVSSVFIFPPKPKDVLTITLTPKVTCVVVDISKDDPEVQFSWFVDDVEVHTAQTQPREEQFNSTFRSVSELPIMHQDWLNGKEFKCRVNSAAFPAPIEKTISKTKGRPKAPQVYTIPPPKEQMAKDKVSLTCMITDFFPEDITVEWQWNGQPAENYKNTQPIMDTDGSYFVYSKLNVQKSNWEAGNTFTCSVLHEGLHNHHTEKSLSHSPGL

SEQ ID NO: 9 - protein, 592 aa, synthetic construct
KELKFVTLVFRHGDRSPIDTFPTDPIKESSWPQGFGQLTQLGMEQHYELGEYIRKRYRKFLNESYKHEQVYIRSTDVDRTLMSAMTNLAALFPPEGVSIWNPILLWQPIPVHTVPLSEDQLLYLPFRNCPRFQELESETLKSEEFQKRLHPYKDFIATLGKLSGLHGQDLFGIWSKVYDPLYCESVHNFTLPSWATEDTMTKLRELSELSLLSLYGIHKQKEKSRLQGGVLVNEILNHMKRATQIPSYKKLIMYSAHDTTVSGLQMALDVYNGLLPPYASCHLTELYFEKGEYFVEMYYRNETQHEPYPLMLPGCSPSCPLERFAELVGPVIPQDWSTECMTTNSHQGTEDSTDSRGGGSVDKKIVPADCGCAPCICAVPEVSSVFIFPPKPKDVLTITLTPKVTCVVVDISKDDPEVQFSWFVDDVEVHTAQTQPREEQFNSTFRSVSELPIMHQDWLNGKEFKCRVNSAAFPLPEEKTISKTKGRPKAPQVYTIPPPKEQMAKDKVSLTCMITDFFPEDITVEWQWNGQPAENYKNTQPIMDTDGSYFVYSKLNVQKSNWEAGNTFTCSVLHEGLHNHHTEKSLSHSPGL

SEQ ID NO: 10 - protein, 597 aa, synthetic construct
KELKFVTLVFRHGDRSPIDTFPTDPIKESSWPQGFGQLTQLGMEQHYELGEYIRKRYRKFLNESYKHEQVYIRSTDVDRTLMSAMTNLAALFPPEGVSIWNPILLWQPIPVHTVPLSEDQLLYLPFRNCPRFQELESETLKSEEFQKRLHPYKDFIATLGKLSGLHGQDLFGIWSKVYDPLYCESVHNFTLPSWATEDTMTKLRELSELSLLSLYGIHKQKEKSRLQGGVLVNEILNHMKRATQIPSYKKLIMYSAHDTTVSGLQMALDVYNGLLPPYASCHLTELYFEKGEYFVEMYYRNETQHEPYPLMLPGCSPSCPLERFAELVGPVIPQDWSTECMTTNSHQGTEDSTDSRGGGSVDKRVEPKSCDKTHTCPPCPAPELLGGPSVFLFPPKPKDTLMISRTPEVTCVVVDVSHEDPEVKFNWYVDGVEVHNAKTKPREEQYNSTYRVVSVLTVLHQDWLNGKEYKCKVSNKALPAPIEKTISKAKGQPREPQVYTLPPSREEMTKNQVSLTCLVKGFYPSDIAVEWESNGQPENNYKTTPPVLDSDGSFFLYSKLTVDKSRWQQGNVFSCSVMHEALHNHYTQKSLSLSPGK

SEQ ID NO: 11 - protein, 20 aa, Virus
MVSAIVLYVLLAAAAHSAFA

SEQ ID NO: 12 - protein, 38 aa, Virus
MLLVNQSHQGFNKEHTSKMVSAIVLYVLLAAAAHSAFA

SEQ ID NO: 13 - protein, 4 aa, synthetic construct
GGGS

SEQ ID NO: 14 - protein, 6 aa, synthetic construct
SRGGGS

SEQ ID NO: 15 - protein, 8 aa, synthetic construct
VRPQGGGS

SEQ ID NO: 16 - protein, 10 aa, synthetic construct
QSLSRSTRGS